European Patent Application EP 4 599 844 A1, published August 13, 2025. Title: CLICK CHEMISTRY HLA POLYPEPTIDES. Applicant: IMMUNEO Therapeutics GmbH. The sequence listing filed with the application follows.

SEQUENCE LISTING (153 sequences)

SEQ ID NO: 1 - protein, 17 aa, synthetic construct
KLVVVGAVGVGKSALTI

SEQ ID NO: 2 - protein, 23 aa, synthetic construct
LANSPDLSHLAYYVTKVKEEDAF

SEQ ID NO: 3 - protein, 17 aa, synthetic construct
LQEFRRFQDPGRIVAIV

SEQ ID NO: 4 - protein, 17 aa, synthetic construct
ETNFKSLFHDLFQKVEE

SEQ ID NO: 5 - protein, 16 aa, synthetic construct
IKPRILGFDTPHYWLC

SEQ ID NO: 6 - protein, 33 aa, synthetic construct
NVGLSAVCTYNLSTAAAYCIHSINLHNFSNSVL

SEQ ID NO: 7 - protein, 22 aa, synthetic construct
MLFSNITPKAAYSPLTGGNMAF

SEQ ID NO: 8 - protein, 37 aa, synthetic construct
KKIRKPRTIYSSLQLQAAAYGIYDALFDIESKVDPSK

SEQ ID NO: 9 - protein, 23 aa, synthetic construct
LPVMLLIVARPVKLAAFPTSLSD

SEQ ID NO: 10 - protein, 16 aa, synthetic construct
LFKDLGLPARTVSTTF

SEQ ID NO: 11 - protein, 10 aa, synthetic construct
SPLTGGNMAF

SEQ ID NO: 12 - protein, 21 aa, synthetic construct
IPDEYGNTALHYAIYNEDKLM

SEQ ID NO: 13 - protein, 35 aa, synthetic construct
LSKNLVAQISALALQLAAYGNSITGIISSVLGHIS

SEQ ID NO: 14 - protein, 22 aa, synthetic construct
SPRQCSSWTLAAYKLAAFPTSL

SEQ ID NO: 15 - protein, 22 aa, synthetic construct
HRCATITHLLAAYYLVLNFNKK

SEQ ID NO: 16 - protein, 15 aa, synthetic construct
RERRVASWAMSFERL

SEQ ID NO: 17 - protein, 21 aa, synthetic construct
QSYPGSASLAAYSGMPRISKL

SEQ ID NO: 18 - protein, 33 aa, synthetic construct
KLVVVGAVGVGKSALTIRQIKIWFQNRRMKWKK

SEQ ID NO: 19 - protein, 39 aa, synthetic construct
LANSPDLSHLAYYVTKVKEEDAFRQIKIWFQNRRMKWKK

SEQ ID NO: 20 - protein, 33 aa, synthetic construct
LQEFRRFQDPGRIVAIVRQIKIWFQNRRMKWKK

SEQ ID NO: 21 - protein, 33 aa, synthetic construct
ETNFKSLFHDLFQKVEERQIKIWFQNRRMKWKK

SEQ ID NO: 22 - protein, 32 aa, synthetic construct
IKPRILGFDTPHYWLCRQIKIWFQNRRMKWKK

SEQ ID NO: 23 - protein, 38 aa, synthetic construct
MLFSNITPKAAYSPLTGGNMAFRQIKIWFQNRRMKWKK

SEQ ID NO: 24 - protein, 31 aa, synthetic construct
RERRVASWAMSFERLRQIKIWFQNRRMKWKK

SEQ ID NO: 25 - protein, 41 aa, synthetic construct
RQRLALEAEKAAYEERGAAEALSVVRQIKIWFQNRRMKWKK

SEQ ID NO: 26 - protein, 37 aa, synthetic construct
IPDEYGNTALHYAIYNEDKLMRQIKIWFQNRRMKWKK

SEQ ID NO: 27 - protein, 32 aa, synthetic construct
LFKDLGLPARTVSTTFRQIKIWFQNRRMKWKK

SEQ ID NO: 28 - protein, 38 aa, synthetic construct
SPRQCSSWTLAAYKLAAFPTSLRQIKIWFQNRRMKWKK

SEQ ID NO: 29 - protein, 38 aa, synthetic construct
HRCATITHLLAAYYLVLNFNKKRQIKIWFQNRRMKWKK

SEQ ID NO: 30 - protein, 32 aa, synthetic construct
KDYSVLYVVPGPVRFQRQIKIWFQNRRMKWKK

SEQ ID NO: 31 - protein, 36 aa, synthetic construct
QSYPGSASLAAYSGMPRISKLRQIKIWFQNRRMKWK

SEQ ID NO: 32 - protein, 34 aa, synthetic construct
AAKALMSAFYTFRYPLSLRQIKIWFQNRRMKWKK

SEQ ID NO: 33 - protein, 49 aa, synthetic construct
ATYLWWVNNQSLPVSPRAAYLLLTASLLTFWNPRQIKIWFQNRRMKWKK

SEQ ID NO: 34 - protein, 36 aa, synthetic construct
DSTPPPGTRVLAMAIYKQSQRQIKIWFQNRRMKWKK

SEQ ID NO: 35 - protein, 36 aa, synthetic construct
EYFMKQMNDARHGGWTTKMDRQIKIWFQNRRMKWKK

SEQ ID NO: 36 - protein, 36 aa, synthetic construct
EYKLVVVGAVGVGKSALTIQRQIKIWFQNRRMKWKK

SEQ ID NO: 37 - protein, 35 aa, synthetic construct
GACRHGDRCSRLHNKPTFSRQIKIWFQNRRMKWKK

SEQ ID NO: 38-39 - skipped (2 entries)

SEQ ID NO: 40 - protein, 36 aa, synthetic construct
HTLYGHTSTVCCMHLHEKRVRQIKIWFQNRRMKWKK

SEQ ID NO: 41 - protein, 36 aa, synthetic construct
HTLYGHTSTVHCMHLHEKRVRQIKIWFQNRRMKWKK

SEQ ID NO: 42 - protein, 36 aa, synthetic construct
ICLTSTVQLIMQLMPFGCLLRQIKIWFQNRRMKWKK

SEQ ID NO: 43 - protein, 40 aa, synthetic construct
IGHKVDAVFMKDGFFYFFHGTRQYRQIKIWFQNRRMKWKK

SEQ ID NO: 44 - protein, 37 aa, synthetic construct
KAISTRDPLSKITEQEKDFLWRQIKIWFQNRRMKWKK

SEQ ID NO: 45 - protein, 35 aa, synthetic construct
KIGDFGLATEKSRWSGSHQRQIKIWFQNRRMKWKK

SEQ ID NO: 46 - protein, 39 aa, synthetic construct
KLVVVGACGVGKSALTIQLIQNHRQIKIWFQNRRMKWKK

SEQ ID NO: 47 - protein, 39 aa, synthetic construct
KLVVVGADGVGKSALTIQLIQNHRQIKIWFQNRRMKWKK

SEQ ID NO: 48 - protein, 34 aa, synthetic construct
KVKIPVAIKTSPKANKEIRQIKIWFQNRRMKWKK

SEQ ID NO: 49 - protein, 35 aa, synthetic construct
LLDILDTAGHEEYSAMRDQRQIKIWFQNRRMKWKK

SEQ ID NO: 50 - protein, 35 aa, synthetic construct
LLGRNSFEVCVCACPGRDRRQIKIWFQNRRMKWKK

SEQ ID NO: 51 - protein, 35 aa, synthetic construct
LLGRNSFEVHVCACPGRDRRQIKIWFQNRRMKWKK

SEQ ID NO: 52 - protein, 35 aa, synthetic construct
LLGRNSFEVLVCACPGRDRRQIKIWFQNRRMKWKK

SEQ ID NO: 53 - protein, 35 aa, synthetic construct
MAQYLSTLLLLLATLAVALRQIKIWFQNRRMKWKK

SEQ ID NO: 54 - protein, 36 aa, synthetic construct
MLPQIPFLLLVSLNLVHGVFRQIKIWFQNRRMKWKK

SEQ ID NO: 55 - protein, 35 aa, synthetic construct
MTEYKLVVVGARGVGKSALRQIKIWFQNRRMKWKK

SEQ ID NO: 56 - protein, 43 aa, synthetic construct
MTEYKLVVVGASGVGKSALTIQLIQNHRQIKIWFQNRRMKWKK

SEQ ID NO: 57 - protein, 35 aa, synthetic construct
NSSCMGGMNQRPILTIITLRQIKIWFQNRRMKWKK

SEQ ID NO: 58 - protein, 35 aa, synthetic construct
NSSCMGGMNWRPILTIITLRQIKIWFQNRRMKWKK

SEQ ID NO: 59 - protein, 35 aa, synthetic construct
PSDQDLLRCCVLTSGIFETRQIKIWFQNRRMKWKK

SEQ ID NO: 60 - protein, 35 aa, synthetic construct
PSDQDLLRCHVLTSGIFETRQIKIWFQNRRMKWKK

SEQ ID NO: 61 - protein, 35 aa, synthetic construct
QHVKITDFGRAKLLGAEEKRQIKIWFQNRRMKWKK

SEQ ID NO: 62 - protein, 35 aa, synthetic construct
RVCACPGRDWRTEEENLRKRQIKIWFQNRRMKWKK

SEQ ID NO: 63 - protein, 35 aa, synthetic construct
SQHMTEVVRHCPHHERCSDRQIKIWFQNRRMKWKK

SEQ ID NO: 64 - protein, 36 aa, synthetic construct
STRDPLSEITKQEKDFLWSHRQIKIWFQNRRMKWKK

SEQ ID NO: 65 - protein, 37 aa, synthetic construct
TEYKLVVVGAAGVGKSALTIQRQIKIWFQNRRMKWKK

SEQ ID NO: 66 - protein, 40 aa, synthetic construct
TIHYNYMCNSSCMGSMNRRPILTIRQIKIWFQNRRMKWKK

SEQ ID NO: 67 - protein, 35 aa, synthetic construct
YGIPFIETSTKTRQRVEDARQIKIWFQNRRMKWKK

SEQ ID NO: 68 - protein, 43 aa, synthetic construct
YKLVVVGAGDVGKSALTIQLIQNHFVDRQIKIWFQNRRMKWKK

SEQ ID NO: 69 - protein, 15 aa, synthetic construct
VAFLGCPGFAGVLQT

SEQ ID NO: 70 - protein, 36 aa, synthetic construct
ESGCEERGAAMIQTVDPAAHRQIKIWFQNRRMKWKK

SEQ ID NO: 71 - protein, 36 aa, synthetic construct
QRQLNTALPQPFREAPAYSNRQIKIWFQNRRMKWKK

SEQ ID NO: 72 - protein, 9 aa, synthetic construct
MLFSNITPK

SEQ ID NO: 73 - protein, 19 aa, synthetic construct
LLFVMESFLLSSALTLCAR

SEQ ID NO: 74 - protein, 15 aa, synthetic construct
SPITSVLSADLFPKA

SEQ ID NO: 75 - protein, 15 aa, synthetic construct
SAANIRALNVPPSLA

SEQ ID NO: 76 - protein, 16 aa, synthetic construct
PQELWHFLTQNLSLPN

SEQ ID NO: 77 - protein, 17 aa, synthetic construct
KKIRKPRTIYSSLQLQA

SEQ ID NO: 78 - protein, 17 aa, synthetic construct
GIYDALFDIESKVDPSK

SEQ ID NO: 79 - protein, 37 aa, synthetic construct
AIYNEDKLMAKALLLYGADIERQIKIWFQNRRMKWKK

SEQ ID NO: 80 - protein, 37 aa, synthetic construct
NFMLNQNVMLSVKGITKNVHTRQIKIWFQNRRMKWKK

SEQ ID NO: 81 - protein, 33 aa, synthetic construct
LTPKKLQCVDLHVISNDRQIKIWFQNRRMKWKK

SEQ ID NO: 82 - protein, 38 aa, synthetic construct
LEKLYLYFNKISKIENLEKLIKRQIKIWFQNRRMKWKK

SEQ ID NO: 83 - protein, 37 aa, synthetic construct
QSYPGSASLAAYSGMPRISKLRQIKIWFQNRRMKWKK

SEQ ID NO: 84 - protein, 41 aa, synthetic construct
PPSNATAETQPIPQKAAYLEAIFLRDWDSLYSHDLDTSADS

SEQ ID NO: 85 - protein, 10 aa, synthetic construct
LANSPDLSHL

SEQ ID NO: 86 - protein, 10 aa, synthetic construct
VTKVKEEDAF

SEQ ID NO: 87 - protein, 15 aa, synthetic construct
NVGLSAVCTYNLSTA

SEQ ID NO: 88 - protein, 15 aa, synthetic construct
CIHSINLHNFSNSVL

SEQ ID NO: 89 - protein, 9 aa, synthetic construct
MLFSNITPK

SEQ ID NO: 90 - protein, 10 aa, synthetic construct
SPLTGGNMAF

SEQ ID NO: 91 - protein, 17 aa, synthetic construct
KKIRKPRTIYSSLQLQA

SEQ ID NO: 92 - protein, 17 aa, synthetic construct
GIYDALFDIESKVDPSK

SEQ ID NO: 93 - protein, 16 aa, synthetic construct
LSKNLVAQISALALQL

SEQ ID NO: 94 - protein, 16 aa, synthetic construct
GNSITGIISSVLGHIS

SEQ ID NO: 95 - protein, 10 aa, synthetic construct
HRCATITHLL

SEQ ID NO: 96 - protein, 9 aa, synthetic construct
YLVLNFNKK

SEQ ID NO: 97 - protein, 9 aa, synthetic construct
QSYPGSASL

SEQ ID NO: 98 - protein, 9 aa, synthetic construct
SGMPRISKL

SEQ ID NO: 99 - protein, 9 aa, synthetic construct
ANSPDLSHL

SEQ ID NO: 100 - protein, 26 aa, synthetic construct
VTKVKEEDAFRQIKIWFQNRRMKWKK

SEQ ID NO: 101 - protein, 17 aa, synthetic construct
ATYLWWVNNQSLPVSPR

SEQ ID NO: 102 - protein, 13 aa, synthetic construct
LLLTASLLTFWNP

SEQ ID NO: 103 - protein, 9 aa, synthetic construct
QSYPGSASL

SEQ ID NO: 104 - protein, 9 aa, synthetic construct
SGMPRISKL

SEQ ID NO: 105 - protein, 15 aa, synthetic construct
PPSNATAETQPIPQK

SEQ ID NO: 106 - protein, 23 aa, synthetic construct
LEAIFLRDWDSLYSHDLDTSADS

SEQ ID NO: 107 - protein, 9 aa, synthetic construct
MLFSNITPK

SEQ ID NO: 108 - protein, 10 aa, synthetic construct
SPLTGGNMAF

SEQ ID NO: 109 - protein, 10 aa, synthetic construct
RQRLALEAEK

SEQ ID NO: 110 - protein, 28 aa, synthetic construct
EERGAAEALSVVRQIKIWFQNRRMKWKK

SEQ ID NO: 111 - protein, 9 aa, synthetic construct
QSYPGSASL

SEQ ID NO: 112 - protein, 25 aa, synthetic construct
SGMPRISKLRQIKIWFQNRRMKWKK

SEQ ID NO: 113 - protein, 15 aa, synthetic construct
PPSNATAETQPIPQK

SEQ ID NO: 114 - protein, 23 aa, synthetic construct
LEAIFLRDWDSLYSHDLDTSADS

SEQ ID NO: 115 - protein, 21 aa, synthetic construct
QSYPGSASLAAYSGMPRISKL

SEQ ID NO: 116 - protein, 15 aa, synthetic construct
RQIKIWFQNRRMKWK

SEQ ID NO: 117 - protein, 10 aa, synthetic construct
LANSPDLSHL

SEQ ID NO: 118 - protein, 10 aa, synthetic construct
VTKVKEEDAF

SEQ ID NO: 119 - protein, 15 aa, synthetic construct
NVGLSAVCTYNLSTA

SEQ ID NO: 120 - protein, 15 aa, synthetic construct
CIHSINLHNFSNSVL

SEQ ID NO: 121 - protein, 9 aa, synthetic construct
MLFSNITPK

SEQ ID NO: 122 - protein, 10 aa, synthetic construct
SPLTGGNMAF

SEQ ID NO: 123 - protein, 16 aa, Drosophila melanogaster
RQIKIWFQNRRMKWKK

SEQ ID NO: 124 - protein, 9 aa, Human immunodeficiency virus 1
RKKRRQRRR

SEQ ID NO: 125 - protein, 13 aa, synthetic construct
GRRRRRRRRRPPQ

SEQ ID NO: 126 - protein, 16 aa, synthetic construct
RKKRRRESRKKRRRES

SEQ ID NO: 127 - protein, 17 aa, synthetic construct
GRPRESGKKRKRKRLKP

SEQ ID NO: 128 - protein, 18 aa, synthetic construct
RKQIKIWFQNRRMKKKWI

SEQ ID NO: 129 - protein, 15 aa, synthetic construct
RQFWIWQNRKWIKIK

SEQ ID NO: 130 - protein, 14 aa, synthetic construct
RQIKVWFQRKWIKK

SEQ ID NO: 131 - protein, 19 aa, synthetic construct
KIQRKIWFQNRRMKVKWKI

SEQ ID NO: 132 - protein, 14 aa, synthetic construct
RKIIWFQNRMKWIK

SEQ ID NO: 133 - protein, 16 aa, synthetic construct
IKVRQWFQNRRMIKWK

SEQ ID NO: 134 - protein, 14 aa, synthetic construct
RQIKIWFQNRKWKK

SEQ ID NO: 135 - protein, 16 aa, synthetic construct
RQIKIWFQNRRMKIKW

SEQ ID NO: 136 - protein, 16 aa, synthetic construct
RKQIKVWFQNRRMKWK

SEQ ID NO: 137 - protein, 17 aa, synthetic construct
NRRMRQIKIWFQKWKIK

SEQ ID NO: 138 - protein, 17 aa, synthetic construct
RQIKIWFVNRKMWKQRI

SEQ ID NO: 139 - protein, 15 aa, synthetic construct
QRIKVWFQRKWKIKK

SEQ ID NO: 140 - protein, 14 aa, synthetic construct
RQIKIWFRMKWKIK

SEQ ID NO: 141 - protein, 19 aa, synthetic construct
QRIKFWIVNRKMKQRIKIW

SEQ ID NO: 142 - protein, 14 aa, synthetic construct
IRQKIWFQNRKMVK

SEQ ID NO: 143 - protein, 16 aa, synthetic construct
RQIKFWIQNRIKWKWK

SEQ ID NO: 144 - protein, 19 aa, synthetic construct
KIRQIWFQNRRMKWKRFKI

SEQ ID NO: 145 - protein, 19 aa, synthetic construct
RQIKIQWFNRRWVKKMWIK

SEQ ID NO: 146 - protein, 16 aa, synthetic construct
RIQKKIWFQNRKWIKM

SEQ ID NO: 147 - protein, 20 aa, synthetic construct
QRKIKIWFQNRRMKVWKIKI

SEQ ID NO: 148 - protein, 13 aa, synthetic construct
AAYRRRRRRRRRR

SEQ ID NO: 149 - protein, 13 aa, synthetic construct
AAYRRRRRRRRRR

SEQ ID NO: 150 - protein, 13 aa, synthetic construct
AAYRRRRRRRRRR

SEQ ID NO: 151 - protein, 12 aa, synthetic construct
AAYRRRRRRRRR

SEQ ID NO: 152 - protein, 12 aa, synthetic construct
AAYRRRRRRRRR

SEQ ID NO: 153 - protein, 12 aa, synthetic construct
AAYRRRRRRRRR